European Patent Application EP 4 386 010 A1, published June 19, 2024. Title: MODIFIED CELL, AND PREPARATION METHOD THEREFOR AND USE THEREOF. Applicant: Cure Genetics Co., Ltd. The sequence listing filed with the application follows.

SEQUENCE LISTING (99 sequences)

SEQ ID NO: 1 - DNA, 19 bp, synthetic construct
  misc_feature 1..19: note = Target sequence of the gRNA targeting B2M-KI
  source 1..19: mol_type = other DNA
ctcacgctggatagcctcc

SEQ ID NO: 2 - RNA, 80 nt, synthetic construct
  misc_feature 1..80: note = gRNA backbone sequence
  source 1..80: mol_type = other RNA
gttttagagctagaaatagcaagttaaaataaggctagtccgttatcaacttgaaaaagtggcaccgagtcggtgctttt

SEQ ID NO: 3 - RNA, 109 nt, synthetic construct
  misc_feature 1..109: note = Targeting gRNA sequence plus backbone sequence of B2M-KI
  source 1..109: mol_type = other RNA
ctcacgctggatagcctccgttttagagctatgctggaaacagcatagcaagttaaaataaggctagtccgttatcaacttgaaaaagtggcaccgagtcggtgctttt

SEQ ID NO: 4 - DNA, 1082 bp, synthetic construct
  misc_feature 1..1082: note = HLA-E restriction-presenting peptide insertion sequence DNA
  source 1..1082: mol_type = other DNA
catatgatcttaatcttctgggtttccgttttctcgaatgaaaaatgcaggtccgagcagttaactggcgggggcaccattagcaagtcacttagcatctctggggccagtctgcaaagcgagggggcagccttaatgtgcctccagcctgaagtcctagaatgagcgcccggtgtcccaagctggggcgcgcaccccagatcggagggcgccgatgtacagacagcaaactcacccagtctagtgcatgccttcttaaacatcacgagactctaagaaaaggaaactgaaaacgggaaagtccctctctctaacctggcactgcgtcgctggcttggagacaggtgacggtccctgcgggccttgtcctgattggctgggcacgcgtttaatataagtggaggcgtcgcgctggcgggcattcctgaagctgacagcattcgggccgagatgtctcgctccgtggccttagctgtgctcgcgctactctctctttctggcctggaggccgttatggctccgcggactgtgctgttaggcggagggggtagcggaggtggcgggtccgggggaggtggctctatccagcgtgagtctctcctaccctcccgctctggtccttcctctcccgctctgcaccctctgtggccctcgctgtgctctctcgctccgtgacttcccttctccaagttctccttggtggcccgccgtggggctagtccagggctggatctcggggaagcggcggggtggcctgggagtggggaagggggtgcgcacccgggacgcgcgctacttgcccctttcggcggggagcaggggagacctttggcctacggcgacgggagggtcgggacaaagtttagggcgtcgataagcgtcagagcgccgaggttgggggagggtttctcttccgctctttcgcggggcctctggctcccccagcgcagctggagtgggggacgggtaggctcgtcccaaaggcgcggcgctgaggtttgtgaacgcgtggaggggcgcttggggtctgggggaggcgtcgcccgggtaagcctgtctgctgcggctctgcttcccttaga

SEQ ID NO: 5 - DNA, 21 bp, synthetic construct
  misc_feature 1..21: note = B2M site-directed insertion detection sequencing primers
  source 1..21: mol_type = other DNA
agcaaactcacccagtctagt

SEQ ID NO: 6 - DNA, 2645 bp, synthetic construct
  misc_feature 1..2645: note = AAV delivery of template DNA for HLA-E restriction peptide NdeI/HpaI
  source 1..2645: mol_type = other DNA
taatgtcaatggaatcaggccagagtttgaattctagtctcttagcctttgtttcccctgtccataaaatgaatgggggtaattctttcctcctacagtttatttatatattcactaattcattcattcatccatccattcgttcattcggtttactgagtacctactatgtgccagcccctgttctagggtggaaactaagagaatgatgtacctagagggcgctggaagctctaaagccctagcagttactgcttttactattagtggtcgtttttttctcccccccgccccccgacaaatcaacagaacaaagaaaattacctaaacagcaaggacatagggaggaacttcttggcacagaactttccaaacactttttcctgaagggatacaagaagcaagaaaggtactctttcactaggaccttctctgagctgtcctcaggatgcttttgggactatttttcttacccagagaatggagaaaccctgcagggaattcccaagctgtagttataaacagaagttctccttctgctaggtagcattcaaagatcttaatcttctgggtttccgttttctcgaatgaaaaatgcaggtccgagcagttaactggcgggggcaccattagcaagtcacttagcatctctggggccagtctgcaaagcgagggggcagccttaatgtgcctccagcctgaagtcctagaatgagcgcccggtgtcccaagctggggcgcgcaccccagatcggagggcgccgatgtacagacagcaaactcacccagtctagtgcatgccttcttaaacatcacgagactctaagaaaaggaaactgaaaacgggaaagtccctctctctaacctggcactgcgtcgctggcttggagacaggtgacggtccctgcgggccttgtcctgattggctgggcacgcgtttaatataagtggaggcgtcgcgctggcgggcattcctgaagctgacagcattcgggccgagatgtctcgctccgtggccttagctgtgctcgcgctactctctctttctggcctggaggccgttatggctccgcggactgtgctgttaggcggagggggtagcggaggtggcgggtccgggggaggtggctctatccagcgtgagtctctcctaccctcccgctctggtccttcctctcccgctctgcaccctctgtggccctcgctgtgctctctcgctccgtgacttcccttctccaagttctccttggtggcccgccgtggggctagtccagggctggatctcggggaagcggcggggtggcctgggagtggggaagggggtgcgcacccgggacgcgcgctacttgcccctttcggcggggagcaggggagacctttggcctacggcgacgggagggtcgggacaaagtttagggcgtcgataagcgtcagagcgccgaggttgggggagggtttctcttccgctctttcgcggggcctctggctcccccagcgcagctggagtgggggacgggtaggctcgtcccaaaggcgcggcgctgaggtttgtgaacgcgtggaggggcgcttggggtctgggggaggcgtcgcccgggtaagcctgtctgctgcggctctgcttcccttagactggagagctgtggacttcgtctaggcgcccgctaagttcgcatgtcctagcacctctgggtctatgtggggccacaccgtggggaggaaacagcacgcgacgtttgtagaatgcttggctgtgatacaaagcggtttcgaataattaacttatttgttcccatcacatgtcacttttaaaaaattataagaactacccgttattgacatctttctgtgtgccaaggactttatgtgctttgcgtcatttaattttgaaaacagttatcttccgccatagataactactatggttatcttctgcctctcacagatgaagaaactaaggcaccgagattttaagaaacttaattacacaggggataaatggcagcaatcgagattgaagtcaagcctaaccagggcttttgcgggagcgcatgccttttggctgtaattcgtgcatttttttttaagaaaaacgcctgccttctgcgtgagattctccagagcaaactgggcggcatgggccctgtggtcttttcgtacagagggcttcctctttggctctttgcctggttgtttccaagatgtactgtgcctcttactttcggttttgaaaacatgagggggttgggcgtggtagcttacgcctgtaatcccagcacttagggaggccgaggcgggaggatggcttgaggtccgtagttgagaccagcctggccaacatggtgaagcctggtctctacaaaaaataataacaaaaattagccgggtgtggtggctcgtgcctgtggtcccagctgctccggtggctgaggcgggaggatctcttgagcttaggcttttgagctatcatggcgccagtgcactccagcgtgggcaacagagcgagaccctgtctctcaaaaaagaaaaaaaaaaaaaaagaaagagaaaagaaaagaaagaaagaagtgaaggtttgtcagtcaggggagttgtaaaaccattaataaagataatccaagatggttaccaagactgttgttaac

SEQ ID NO: 7 - RNA, 109 nt, synthetic construct
  misc_feature 1..109: note = Targeting TRAC-KO sgRNA
  source 1..109: mol_type = other RNA
gagtctctcagctggtacagttttagagctatgctggaaacagcatagcaagttaaaataaggctagtccgttatcaacttgaaaaagtggcaccgagtcggtgctttt

SEQ ID NO: 8 - DNA, 1461 bp, synthetic construct
  misc_feature 1..1461: note = DNA sequence of CJP
  source 1..1461: mol_type = other DNA
atggccttaccagtgaccgccttgctcctgccgctggccttgctgctccacgccgccaggccggacatccagatgacacagactacatcctccctgtctgcctctctgggagacagagtcaccatcagttgcagggcaagtcaggacattagtaaatatttaaattggtatcagcagaaaccagatggaactgttaaactcctgatctaccatacatcaagattacactcaggagtcccatcaaggttcagtggcagtgggtctggaacagattattctctcaccattagcaacctggagcaagaagatattgccacttacttttgccaacagggtaatacgcttccgtacacgttcggaggggggaccaagctggagatcacaggtggcggtggctcgggcggtggtgggtcgggtggcggcggatctgaggtgaaactgcaggagtcaggacctggcctggtggcgccctcacagagcctgtccgtcacatgcactgtctcaggggtctcattacccgactatggtgtaagctggattcgccagcctccacgaaagggtctggagtggctgggagtaatatggggtagtgaaaccacatactataattcagctctcaaatccagactgaccatcatcaaggacaactccaagagccaagttttcttaaaaatgaacagtctgcaaactgatgacacagccatttactactgtgccaaacattattactacggtggtagctatgctatggactactggggccaaggaacctcagtcaccgtctcctcaaccacgacgccagcgccgcgaccaccaacaccggcgcccaccatcgcgtcgcagcccctgtccctgcgcccagaggcgtgccggccagcggcggggggcgcagtgcacacgagggggctggacttcgcctgtgatatctacatctgggcgcccttggccgggacttgtggggtccttctcctgtcactggttatcaccctttactgcaaacggggcagaaagaaactcctgtatatattcaaacaaccatttatgagaccagtacaaactactcaagaggaagatggctgtagctgccgatttccagaagaagaagaaggaggatgtgaactgagagtgaagttcagcaggagcgcagacgcccccgcgtacaagcagggccagaaccagctctataacgagctcaatctaggacgaagagaggagtacgatgttttggacaagagacgtggccgggaccctgagatggggggaaagccgagaaggaagaaccctcaggaaggcctgtacaatgaactgcagaaagataagatggcggaggcctacagtgagattgggatgaaaggcgagcgccggaggggcaaggggcacgatggcctttaccagggtctcagtacagccaccaaggacacctacgacgcccttcacatgcaggccctgccccctcgctaa

SEQ ID NO: 9 - protein, 24 aa, synthetic construct
  REGION 1..24: note = Protein sequence of HLA-E-restricted presenting peptide-linker
VMAPRTVLLGGGGSGGGGSGGGGS

SEQ ID NO: 10 - DNA, 22 bp, synthetic construct
  misc_feature 1..22: note = PCR upstream primers for amplification of homologous recombinant DNA
  source 1..22: mol_type = other DNA
atcttaatcttctgggtttccg

SEQ ID NO: 11 - DNA, 22 bp, synthetic construct
  misc_feature 1..22: note = PCR downstream primers for amplification of homologous recombinant DNA
  source 1..22: mol_type = other DNA
tctaagggaagcagagccgcag

SEQ ID NO: 12 - DNA, 76 bp, synthetic construct
  misc_feature 1..76: note = Nucleotide sequence of HLA-E restriction-presenting peptide-linker
  source 1..76: mol_type = other DNA
ggccgttatggctccgcggactgtgctgttaggcggagggggtagcggaggtggcgggtccgggggaggtggctct

SEQ ID NO: 13 - RNA, 19 nt, synthetic construct
  misc_feature 1..19: note = Targeting the gRNA sequence of B2M-KI
  source 1..19: mol_type = other RNA
ctcacgctggatagcctcc

SEQ ID NO: 14 - protein, 119 aa, synthetic construct
  REGION 1..119: note = B2M protein containing signal peptide
MSRSVALAVLALLSLSGLEAIQRTPKIQVYSRHPAENGKSNFLNCYVSGFHPSDIEVDLLKNGERIEKVEHSDLSFSKDWSFYLLYYTEFTPTEKDEYACRVNHVTLSQPKIVKWDRDM

SEQ ID NO: 15 - protein, 99 aa, synthetic construct [sequence omitted]

SEQ ID NO: 16 - protein, 20 aa, synthetic construct
  REGION 1..20: note = B2M signal peptide
MSRSVALAVLALLSLSGLEA

SEQ ID NO: 17 - skipped

SEQ ID NO: 18 - protein, 10 aa, synthetic construct
  REGION 1..10: note = 1st Presenting peptide
YLLPRRGPRL

SEQ ID NO: 19 - protein, 9 aa, synthetic construct
  REGION 1..9: note = 2nd Presentation peptide
ALALVRMLI

SEQ ID NO: 20 - protein, 9 aa, synthetic construct
  REGION 1..9: note = 3rd Presentation peptide
AISPRTLNA

SEQ ID NO: 21 - protein, 9 aa, synthetic construct
  REGION 1..9: note = 4th Presentation peptide
QMRPVSRVL

SEQ ID NO: 22 - protein, 9 aa, synthetic construct
  REGION 1..9: note = 5th Presentation peptide
SQQPYLQLQ

SEQ ID NO: 23 - protein, 9 aa, synthetic construct
  REGION 1..9: note = 6th Presentation peptide
VTAPRTLLL

SEQ ID NO: 24 - protein, 9 aa, synthetic construct
  REGION 1..9: note = 7th Presentation peptide
VTAPRTVLL

SEQ ID NO: 25 - protein, 9 aa, synthetic construct
  REGION 1..9: note = 8th Presentation peptide
VTAPRTLVL

SEQ ID NO: 26 - protein, 9 aa, synthetic construct
  REGION 1..9: note = 9th Presentation peptide
VMAPQALLL

SEQ ID NO: 27 - protein, 9 aa, synthetic construct
  REGION 1..9: note = 10th Presentation peptide
VMAPRALLL

SEQ ID NO: 28 - protein, 9 aa, synthetic construct
  REGION 1..9: note = 11th Presentation peptide
VMAPRTLTL

SEQ ID NO: 29 - protein, 9 aa, synthetic construct
  REGION 1..9: note = 12th Presentation peptide
VMAPRTLFL

SEQ ID NO: 30 - protein, 9 aa, synthetic construct
  REGION 1..9: note = 13th Presentation peptide
VMAPRTLVL

SEQ ID NO: 31 - protein, 9 aa, synthetic construct
  REGION 1..9: note = 14th Presentation peptide
VMAPRTLIL

SEQ ID NO: 32 - protein, 9 aa, synthetic construct
  REGION 1..9: note = 15th Presentation peptide
IMAPRTLVL

SEQ ID NO: 33 - protein, 9 aa, synthetic construct
  REGION 1..9: note = 16th Presentation peptide
VMAPRTLLL

SEQ ID NO: 34 - protein, 9 aa, synthetic construct
  REGION 1..9: note = 17th Presentation peptide
VMPPRTLLL

SEQ ID NO: 35 - protein, 9 aa, synthetic construct
  REGION 1..9: note = 18th Presentation peptide
VMAPRTVLL

SEQ ID NO: 36 - protein, 9 aa, synthetic construct
  REGION 1..9: note = 19th Presentation peptide
VMAPRSLLL

SEQ ID NO: 37 - protein, 9 aa, synthetic construct
  REGION 1..9: note = 20th Presentation peptide
VMAPRSLIL

SEQ ID NO: 38 - protein, 9 aa, synthetic construct
  REGION 1..9: note = 21st Presenting peptide
VMTPRTLVL

SEQ ID NO: 39 - protein, 9 aa, synthetic construct
  REGION 1..9: note = 22nd presentation peptide
VMAPRILIL

SEQ ID NO: 40 - protein, 9 aa, synthetic construct
  REGION 1..9: note = 23rd presentation peptide
AMAPRTLIL

SEQ ID NO: 41 - protein, 9 aa, synthetic construct
  REGION 1..9: note = 24th Presenting peptide
VIAPRTLVL

SEQ ID NO: 42 - protein, 9 aa, synthetic construct
  REGION 1..9: note = 25th Presenting peptide
VMAPQSLLL

SEQ ID NO: 43 - protein, 9 aa, synthetic construct
  REGION 1..9: note = 26th Presenting peptide
VMAPRTFVL

SEQ ID NO: 44 - protein, 9 aa, synthetic construct
  REGION 1..9: note = 27th Presenting peptide
VMTPRTLIL

SEQ ID NO: 45 - protein, 9 aa, synthetic construct
  REGION 1..9: note = 28th Presenting peptide
VTAPRTLIL

SEQ ID NO: 46 - protein, 9 aa, synthetic construct
  REGION 1..9: note = 29th Presenting peptide
VMAPWTLLL

SEQ ID NO: 47 - protein, 9 aa, synthetic construct
  REGION 1..9: note = 30th Presenting peptide
VMVPRSLIL

SEQ ID NO: 48 - protein, 9 aa, synthetic construct
  REGION 1..9: note = 31st presentation peptide
AMAPRTLVL

SEQ ID NO: 49 - protein, 9 aa, synthetic construct
  REGION 1..9: note = 32nd presentation peptide
VIAPRTLIL

SEQ ID NO: 50 - protein, 9 aa, synthetic construct
  REGION 1..9: note = 33rd presentation peptide
VIAPRTLLL

SEQ ID NO: 51 - protein, 9 aa, synthetic construct
  REGION 1..9: note = 34th presentation peptide
VLAPRTLIL

SEQ ID NO: 52 - protein, 9 aa, synthetic construct
  REGION 1..9: note = 35th presentation peptide
VMALRTLIL

SEQ ID NO: 53 - protein, 9 aa, synthetic construct
  REGION 1..9: note = 36th presentation peptide
VMAPRGLIL

SEQ ID NO: 54 - protein, 9 aa, synthetic construct
  REGION 1..9: note = 37th presentation peptide
VMAPRNLIL

SEQ ID NO: 55 - protein, 9 aa, synthetic construct
  REGION 1..9: note = 38th presentation peptide
VMAPRTLFV

SEQ ID NO: 56 - protein, 9 aa, synthetic construct
  REGION 1..9: note = 39th presentation peptide
VMAPRTLLM

SEQ ID NO: 57 - protein, 9 aa, synthetic construct
  REGION 1..9: note = 40th presentation peptide
VMAPRTLVM

SEQ ID NO: 58 - protein, 9 aa, synthetic construct
  REGION 1..9: note = 41st presentation peptide
VMAPRTSLL

SEQ ID NO: 59 - protein, 9 aa, synthetic construct
  REGION 1..9: note = 42nd presentation peptide
VMAPRTSVL

SEQ ID NO: 60 - protein, 9 aa, synthetic construct
  REGION 1..9: note = 43rd presentation peptide
VMAPWTLIL

SEQ ID NO: 61 - protein, 9 aa, synthetic construct
  REGION 1..9: note = 44th presentation peptide
VMAPWTLVL

SEQ ID NO: 62 - protein, 9 aa, synthetic construct
  REGION 1..9: note = 45th presentation peptide
VMDPRTLLL

SEQ ID NO: 63 - protein, 9 aa, synthetic construct
  REGION 1..9: note = 46th presentation peptide
VMGPRTLIL

SEQ ID NO: 64 - protein, 9 aa, synthetic construct
  REGION 1..9: note = 47th presentation peptide
VMGPRTLLL

SEQ ID NO: 65 - protein, 9 aa, synthetic construct
  REGION 1..9: note = 48th presentation peptide
VMVPQTLIL

SEQ ID NO: 66 - protein, 9 aa, synthetic construct
  REGION 1..9: note = 49th presentation peptide
VMVPRTLLL

SEQ ID NO: 67 - protein, 9 aa, synthetic construct
  REGION 1..9: note = 50th presentation peptide
VVAPRTLIL

SEQ ID NO: 68 - protein, 9 aa, synthetic construct
  REGION 1..9: note = 51st presentation peptide
VVAPRTLLL

SEQ ID NO: 69 - protein, 9 aa, synthetic construct
  REGION 1..9: note = 52nd presentation peptide
VMVPRTLIL

SEQ ID NO: 70 - protein, 9 aa, synthetic construct
  REGION 1..9: note = 53rd presentation peptide
VMATRTLLL

SEQ ID NO: 71 - protein, 5 aa, synthetic construct
  REGION 1..5: note = 1st linker
GGGGS

SEQ ID NO: 72 - protein, 5 aa, synthetic construct
  REGION 1..5: note = 2nd linker
QQQQG

SEQ ID NO: 73 - protein, 5 aa, synthetic construct
  REGION 1..5: note = 3rd linker
SSSSG

SEQ ID NO: 74 - protein, 5 aa, synthetic construct
  REGION 1..5: note = 4th linker
EAAAK

SEQ ID NO: 75 - protein, 16 aa, synthetic construct
  REGION 1..16: note = 5th linker
AKTTPKLEEGEFSEAR

SEQ ID NO: 76 - protein, 17 aa, synthetic construct
  REGION 1..17: note = 6th linker
AKTTPKLEEGEFSEARV

SEQ ID NO: 77 - protein, 9 aa, synthetic construct
  REGION 1..9: note = 7th linker
AKTTPKLGG

SEQ ID NO: 78 - protein, 6 aa, synthetic construct
  REGION 1..6: note = 12th linker
RADAAP

SEQ ID NO: 79 - protein, 9 aa, synthetic construct
  REGION 1..9: note = 13th linker
RADAAPTVS

SEQ ID NO: 80 - protein, 12 aa, synthetic construct
  REGION 1..12: note = 14th linker
RADAAAAGGPGS

SEQ ID NO: 81 - protein, 27 aa, synthetic construct
  REGION 1..27: note = 15th linker
RADAAAAGGGGSGGGGSGGGGSGGGGS

SEQ ID NO: 82 - protein, 6 aa, synthetic construct
  REGION 1..6: note = 16th linker
SAKTTP

SEQ ID NO: 83 - protein, 10 aa, synthetic construct
  REGION 1..10: note = 17th linker
SAKTTPKLGG

SEQ ID NO: 84 - protein, 18 aa, synthetic construct
  REGION 1..18: note = 18th linker
SAKTTPKLEEGEFSEARV

SEQ ID NO: 85 - protein, 5 aa, synthetic construct
  REGION 1..5: note = 19th linker
ADAAP

SEQ ID NO: 86 - protein, 12 aa, synthetic construct
  REGION 1..12: note = 20th linker
ADAAPTVSIFPP

SEQ ID NO: 87 - protein, 5 aa, synthetic construct
  REGION 1..5: note = 21st linker
TVAAP

SEQ ID NO: 88 - protein, 12 aa, synthetic construct
  REGION 1..12: note = 22nd Linker
TVAAPSVFIFPP

SEQ ID NO: 89 - protein, 6 aa, synthetic construct
  REGION 1..6: note = 23rd Linker
QPKAAP

SEQ ID NO: 90 - protein, 13 aa, synthetic construct
  REGION 1..13: note = 24th Linker
QPKAAPSVTLFPP

SEQ ID NO: 91 - protein, 6 aa, synthetic construct
  REGION 1..6: note = 25th Linker
AKTTPP

SEQ ID NO: 92 - protein, 13 aa, synthetic construct
  REGION 1..13: note = 26th Linker
AKTTPPSVTPLAP

SEQ ID NO: 93 - protein, 6 aa, synthetic construct
  REGION 1..6: note = 27th Linker
AKTTAP

SEQ ID NO: 94 - protein, 13 aa, synthetic construct
  REGION 1..13: note = 28th Linker
AKTTAPSVYPLAP

SEQ ID NO: 95 - protein, 6 aa, synthetic construct
  REGION 1..6: note = 29th Linker
ASTKGP

SEQ ID NO: 96 - protein, 13 aa, synthetic construct
  REGION 1..13: note = 30th Linker
ASTKGPSVFPLAP

SEQ ID NO: 97 - protein, 14 aa, synthetic construct
  REGION 1..14: note = 31st Linker
GGGGSGGSGSGGGS

SEQ ID NO: 98 - protein, 20 aa, synthetic construct
  REGION 1..20: note = 32nd Linker
GGGGSGGGGSGGGGSGGGGS

SEQ ID NO: 99 - protein, 15 aa, synthetic construct
  REGION 1..15: note = 33rd Linker
GGGGSGGGGSGGGGS